European Patent Specification EP 3 608 331 B1, published January 3, 2024. Title: Peptide for Inhibiting Biofilm. Applicant: Seoul National University R and DB Foundation Nano Intelligent Biomedical Engineering Corporation. co. Ltd. The sequence listing filed with the application follows.

SEQUENCE LISTING (1 sequence)

SEQ ID NO: 1 - protein, 15 aa, Artificial Sequence
  Peptide fragment derived from Human beta-defensin-3
GKCSTRGRKCCRRKK